European Patent Specification EP 3 104 852 B1, published August 14, 2024. Title: Compositions and Methods for Treating Aging and Age-Related Diseases and Symptoms. Applicant: The Regents of the University of California. The sequence listing filed with the application follows.

SEQUENCE LISTING (7 sequences)

SEQ ID NO: 1 - DNA, 22 bp, Caenorhabditis elegans
tgacaacattttccgtttcacc

SEQ ID NO: 2 - DNA, 22 bp, Caenorhabditis elegans
aaatagcctggacggatgtgat

SEQ ID NO: 3 - DNA, 22 bp, Caenorhabditis elegans
gatccgagacaagatgaacgtg

SEQ ID NO: 4 - DNA, 22 bp, Caenorhabditis elegans
acaatttggaacccaaccaatc

SEQ ID NO: 5 - DNA, 22 bp, Caenorhabditis elegans
tgatttggaccgagaattcctt

SEQ ID NO: 6 - DNA, 22 bp, Caenorhabditis elegans
ggatcagacgtttgaacagcac

SEQ ID NO: 7 - protein, 50 aa, Homo sapiens
IMNVIGEPIDERGPIKTKQFAPIHAEAPEFMEMSVEQEILVTGIKVVDLL